European Patent Application EP 4 218 774 A1, published August 2, 2023. Title: METHOD FOR ISOLATION AND PURIFICATION OF MICROVESICLES FROM CELL CULTURE SUPERNATANTS AND BIOLOGICAL FLUIDS. Applicant: UNIVERSITY OF MIAMI. Application EP 23155007.0, filed February 5, 2023. The sequence listing filed with the application follows.

SEQUENCE LISTING (4 sequences)

SEQ ID NO: 1 - DNA, 24 bp, synthetic construct
  misc_feature 1..24: note = Primer
  source 1..24: mol_type = other DNA
agacctcacagtaaaaataggtga

SEQ ID NO: 2 - DNA, 20 bp, synthetic construct
  misc_feature 1..20: note = Primer
  source 1..20: mol_type = other DNA
ctgatgggacccactccatc

SEQ ID NO: 3 - DNA, 25 bp, synthetic construct
  misc_feature 1..25: note = Primer
  source 1..25: mol_type = other DNA
gaagacctcacagtaaaaataggtg

SEQ ID NO: 4 - DNA, 20 bp, synthetic construct
  misc_feature 1..20: note = Primer
  source 1..20: mol_type = other DNA
ctgatgggacccactccatc